European Patent Application EP 4 696 701 A1, published February 18, 2026. Title: 蛋白质、包含其的培养基及其应用. Applicant: 张菁. The sequence listing filed with the application follows.

SEQUENCE LISTING (50 sequences)

SEQ ID NO: 1 - protein, 66 aa, synthetic construct
TKVHNTEPVENARIEPPDTGLYYDEYLKQVIEVLETDPHFREKLQKADIEEIRSGRLSQELDLVSH

SEQ ID NO: 2 - protein, 66 aa, synthetic construct
TKVHNVEPVESARIEPPDTGLYYDEYLKQVIEVLETDPHFREKLQKADIEEIRSGRLSQELDLVSH

SEQ ID NO: 3 - protein, 66 aa, synthetic construct
TKVHNIEPVESAKMEPPDTGLYYDEYLKQVIDVLETDQHFREKLQKADIEEIRSGRLSKELDLVSH

SEQ ID NO: 4 - protein, 66 aa, synthetic construct
TKVGNPEPVESAKIDPPDTGLYYNEYLRQVIDVLETDNHFREKLQKADIEEIKSGKLSKELDLVSH

SEQ ID NO: 5 - protein, 66 aa, synthetic construct
TKVQNTQPVESARIEPPDTGLYYDEYLKQVIDVLETDQHFREKLQKADIEEIKSGRLSKELDLVSH

SEQ ID NO: 6 - protein, 66 aa, synthetic construct
TKVHNTEPVESAKIEPPDTGLYYDEYLKQVIDVLETDQHFREKLQKADIEEIRSGRLSKELDLVSH

SEQ ID NO: 7 - protein, 66 aa, synthetic construct
TKVQNTQPVESSKIEPPDTGLYYDEYLKQVIDVLETDKHFREKLQKADIEEIKSGRLSKELDLVSH

SEQ ID NO: 8 - protein, 66 aa, synthetic construct
TKVQNIHPVESAKIESPDTGLYYDEYLKQVIDVLETDKHFREKLQKADIEEIKSGRLSKELDLVSH

SEQ ID NO: 9 - protein, 66 aa, synthetic construct
TKVQNTHPVESAKIGPPDTGLYYDEYLKQVIEVLETDQHFREKLQKADVEEIKSGRLSKELDLVSH

SEQ ID NO: 10 - protein, 66 aa, synthetic construct
TKVQNTHPVESAKIGPPDTGLYYDEYLKQVIDVLETDRHFREKLQKADVEEIKSGRLSKELDLVSH

SEQ ID NO: 11 - protein, 66 aa, synthetic construct
TKVQNIHPVESAKIEPPDTGLYYDEYLKQVIDVLETDKHFREKLQKADIEEIKSGRLSKELDLVSH

SEQ ID NO: 12 - protein, 66 aa, synthetic construct
TKVKNTQPVDSARIEPPDTGLYYDEYLKQVIDVLETDNHFREKLQKADIEEIKSGRLSKELDLVSH

SEQ ID NO: 13 - protein, 66 aa, synthetic construct
TKVKNTEPVESAKIEPPDTGLYYDEYLKQVIDVLETDNHFREKLQKADIEEIKSGKLSKELDLVSH

SEQ ID NO: 14 - protein, 66 aa, synthetic construct
TKVKNIQPVDSAKIEPPDTGLYYDEYLKQVIDVLETDNHFREKLQKADIEEIKSGRLSKELDLVSH

SEQ ID NO: 15 - protein, 66 aa, synthetic construct
TKVKNNQPVDSAKIEPPDTGLYYDEYLKQVIDVLETDNHFREKLQKADIEEIKSGRLSKELDLVSH

SEQ ID NO: 16 - protein, 66 aa, synthetic construct
TKVENAQPMDSAKIEPPDTGLYYDEYLKQVIDVLETDNHFREKLQKADIEEIKSGRLSKELDLVSH

SEQ ID NO: 17 - protein, 66 aa, synthetic construct
TKVQNTHPVESAKIEPPDTGLYYDTYLKQVIDVLETDQHFREKLQKADIEEIKSGRLSKELDLVSH

SEQ ID NO: 18 - protein, 66 aa, synthetic construct
TKVKNPQPVDSAKIEPPDTGLYYDEYLKQVIDVLETDNHFREKLQKADIEEIKSGRLSKELDLVSH

SEQ ID NO: 19 - protein, 66 aa, synthetic construct
TKVKNTQPMDSAKIEPPDTGLYCDEYLKQVIDVLETDNHFREKLQKADIEEIKSGRLSRELDLVSH

SEQ ID NO: 20 - protein, 66 aa, synthetic construct
TKVKDIPNVEGEKIETPDTGLYYDEYLRQVIDVLETDKHFREKLQNADIEEIKSGKLSKELDLVSH

SEQ ID NO: 21 - protein, 66 aa, synthetic construct
TKVQNTQPVESAKIEPPDTGLYYDEYLKQVIDVLETDKHFREKLQKADIEEIKSGRLSKELDLVSH

SEQ ID NO: 22 - protein, 65 aa, synthetic construct
TKVKTQPVDSAKIEPPDTGLYYDEYLKQVIDVLETDNHFREKLQKADIEEIKSGRLSKELDLVSH

SEQ ID NO: 23 - protein, 66 aa, synthetic construct
TKVKHTQPVESAKIEAPDTGLYYDEYLKQVIDVLETDNHFREKLQKADIEEIKSGRLSKELDLVSH

SEQ ID NO: 24 - protein, 66 aa, synthetic construct
TKVKNTQPVDSAKIEPPGTGLYYDEYLKQVIDVLETDNYFREKLQKADIEEIKSGRLSKELDLVSH

SEQ ID NO: 25 - protein, 66 aa, synthetic construct
TKVQGEPHVEGAKIETPDTGLYYDEYLKQVIDVLETDKHFREKLQTADIEEIKSGKLSKELDLVSH

SEQ ID NO: 26 - protein, 66 aa, synthetic construct
TKVENAQPVDSAKIEPPDTGLYYDEYLKQVIDVLETDNHFREKLQKADIEEIKSGRLSKELDLVSH

SEQ ID NO: 27 - protein, 66 aa, synthetic construct
TKVKNNPPVDSAKIEPPDTGLYYDEYLKQVIDVLETDNHFREKLQKADIEEIKSGRLSKELDLVSH

SEQ ID NO: 28 - protein, 66 aa, synthetic construct
TKVKSPEPVESAKIEPPDTGLYYDEYLKQVIDVLETDKHFREKLQKADIEEIKSGRLSKELDLVSH

SEQ ID NO: 29 - protein, 66 aa, synthetic construct
TKVHNVEPVESAKIEPPDTGLYYDEYLKQVIDVLETDQHFREKLQKADIEEIRNGRLSKELDFVSH

SEQ ID NO: 30 - protein, 66 aa, synthetic construct
TKVKSAQPVDSAKIEPPDTGLYYDEYLKQVIDVLETDSHFREKLQKADIEEIKSGRLSKELDLVSH

SEQ ID NO: 31 - protein, 66 aa, synthetic construct
TKVKAAQPVDSAKIEPPDTGLYYDEYLKQVIDVLETDSHFREKLQKADIEEIKSGRLSKELDLVSH

SEQ ID NO: 32 - protein, 66 aa, synthetic construct
TKVHNAEPVESARIEPPDTGLYYDEYLKQVIEVLETDPHFREKLQKADIEEIRSGRLSQELDLVSH

SEQ ID NO: 33 - protein, 66 aa, synthetic construct
TKVQNTEPVESAKIEPPDTGLYYDEYLKQVIDVLETDKHFREKLQKADIEEIKSGRLSKELDLVSH

SEQ ID NO: 34 - protein, 66 aa, synthetic construct
TKVKGAQPVDSAKIEPPDTGLYYDEYLKQVIDVLETDNHFREKLQKADIEEIKSGRLSKELDLVSH

SEQ ID NO: 35 - protein, 66 aa, synthetic construct
TKVKNTHPVDSAKIEPPDTGLYYDEYLKQVIDVLETDNHFREKLQKADIEEIKSGRLSKELDLVSH

SEQ ID NO: 36 - protein, 66 aa, synthetic construct
TKVKNAQPVDSAKIEPPDTGLYYDEYLKQVIDVLETDNHFREKLQKADIEEIKSGKLSKELDLVSH

SEQ ID NO: 37 - protein, 66 aa, synthetic construct
TKVKNPHPVDSAKIEPPDTGLYYDEYLKQVIDVLETDNHFREKLQKADIEEIKSGRLSKELDLVSH

SEQ ID NO: 38 - protein, 65 aa, synthetic construct
TKVQNIPVESAKIEPPDTGLYYDEYLKQVIDVLETDKHFREKLQKADIEEIKSGRLSKELDLVSH

SEQ ID NO: 39 - protein, 66 aa, synthetic construct
TKVHNTEPVESARIDPPDTGLYYDEYLKQVIDVLETDQHFREKLQKADIEEIRSGRLSKELDLVSH

SEQ ID NO: 40 - protein, 66 aa, synthetic construct
TKVQNIHPVESAKIDPPDTGLYYDEYLKQVIDVLETDKHFREKLQKADIEEIKSGRLSKELDLVSH

SEQ ID NO: 41 - protein, 66 aa, synthetic construct
TKVQNTHPVESAKIEPPDTGLYYDEYLKQVIDVLETDKHFREKLQKADIEEIKSGRLSKELDLVSH

SEQ ID NO: 42 - protein, 66 aa, synthetic construct
TKVKDTPDVEGEKIEPPDTGLYYDEYLKQVIDVLETDQHFREKLQNADIEEIKNGKLSKELDLVSH

SEQ ID NO: 43 - protein, 66 aa, synthetic construct; identical to SEQ ID NO: 25

SEQ ID NO: 44 - protein, 66 aa, synthetic construct
TKVKNPHPMDSAKIEPPDTGLYYDEYLKQVIDVLETDNHFREKLQKADIEEIKSGRLSKELDLVSH

SEQ ID NO: 45 - protein, 66 aa, synthetic construct
TKVQNIPPVESAKIEPPDTGLYYDEYLKQVIDVLETDQHFREKLQKADIEEIKSGKLSKELDLVSH

SEQ ID NO: 46 - protein, 66 aa, synthetic construct
TKVKTTQPVDSAKIEPPDTGLYYDEYLKQVIDVLETDSHFREKLQKADIEEIKSGRLSKELDLVSH

SEQ ID NO: 47 - protein, 66 aa, synthetic construct
TKVKNTQPVDSAKIEPPDTGLYYDEYLKQVIDVLETDNHFREKLQKADIEEIKSGRLSKELDLVSH

SEQ ID NO: 48 - protein, 66 aa, synthetic construct
TKVHNTEPVENARIEPPDTGLYYDEYLKQVIEVLETDPHFREKLQKADIEEIKSGRLSKELDLVSH

SEQ ID NO: 49 - protein, 67 aa, synthetic construct
STKVHNTEPVENARIEPPDTGLYYDEYLKQVIEVLETDPHFREKLQKADIEEIKSGRLSKELDLVSH

SEQ ID NO: 50 - protein, 72 aa, synthetic construct
STKVHNTEPVENARIEPPDTGLYYDEYLKQVIEVLETDPHFREKLQKADIEEIKSGRLSKELDLVSHGLVPR